European Patent Specification EP 3 397 275 B1, published October 9, 2024. Title: Nucleic acid molecules encoding for chimeric CSPG4 proteins and therapeutic uses thereof. Applicant: Universita' degli Studi di Torino The General Hospital Corporation. The sequence listing filed with the application follows.

SEQUENCE LISTING (23 sequences)

SEQ ID NO: 1 - DNA, 33 bp, artificial
  primer
ccggaattcgccatgcagtccgggccgcggccc

SEQ ID NO: 2 - DNA, 28 bp, artificial
  primer
ggtctagagacaccatcaccaggtagcc

SEQ ID NO: 3 - DNA, 33 bp, artificial
  primer
ccggaattcgcctgcttgaagtgcaggcatccg

SEQ ID NO: 4 - DNA, 29 bp, artificial
  primer
ggtctagatcacacccagtactggccgtt

SEQ ID NO: 5 - DNA, 6936 bp, artificial
  HuDo-CSPG4-1
gaattcatgcagtccgggccgcggcccccacttccagcccccggcctggccttggctttgaccctgactatgttggccagacttgcatccgcggcttccttcttcggtgagaaccacctggaggtgcctgtggccacggctctgaccgacatagacctgcagctgcagttctccacgtcccagcccgaagccctccttctcctggcagcaggcccagctgaccacctcctgctgcagctctactctggacgcctgcaggtcagacttgttctgggccaggaggagctgaggctgcagactccagcagagacgctgctgagtgactccatcccccacactgtggtgctgactgtcgtagagggctgggccacgttgtcagtcgatgggtttctgaacgcctcctcagcagtcccaggagcccccctagaggtcccctatgggctctttgttgggggcactgggacccttggcctgccctacctgaggggaaccagccgacccctgaggggttgcctccatgcagccaccctcaatggccgcagcctcctccggcctctgacccccgatgtgcatgagggctgtgctgaagagttttctgccagtgatgatgtggccctgggcttctctgggccccactctctggctgccttccctgcctggggcactcaggacgaaggaaccctagagtttacactcaccacacagagccggcaggcacccttggccttccaggcagggggccggcgtggggacttcatctatgtggacatatttgagggccacctgcgggccgtggtggagaagggccagggtaccgtattgctccacaacagtgtgcctgtggccgatgggcagccccatgaggtcagtgtccacatcaatgctcaccggctggaaatctccgtggaccagtaccctacgcatacttcgaaccgaggagtcctcagctacctggagccacggggcagtctccttctcggggggctggatgcagaggcctctcgtcacctccaggaacaccgcctgggcctgacaccagaggccaccaatgcctccctgctgggctgcatggaagacctcagtgtcaatggccagaggcgggggctgcgggaagctttgctgacgcgcaacatggcagccggctgcaggctggaggaggaggagtatgaggacgatgcctatggacattatgaagctttctccaccctggcccctgaggcttggccagccatggagctgcctgagccatgcgtgcctgagccagggctgcctcctgtctttgccaatttcacccagctgctgactatcagcccactggtggtggccgaggggggcacagcctggcttgagtggaggcatgtgcagcccacgctggacctgatggaggctgagctgcgcaaatcccaggtgctgttcagcgtgacccgaggggcacgccatggcgagctcgagctggacatcccgggagcccaggcacgaaaaatgttcaccctcctggacgtggtgaaccgcaaggcccgcttcatccacgatggctctgaggacacctccgaccagctggtgctggaggtgtcggtgacggctcgggtgcccatgccctcatgccttcggaggggccaaacatacctcctgcccatccaggtcaaccctgtcaatgacccaccccacatcatcttcccacatggcagcctcatggtgatcctggaacacacgcagaagccgctggggcctgaggttttccaggcctatgacccggactctgcctgtgagggcctcaccttccaggtccttggcacctcctctggcctccccgtggagcgccgagaccagcctggggagccggcgaccgagttctcctgccgggagttggaggccggcagcctagtctatgtccaccgcggtggtcctgcacaggacttgacgttccgggtcagcgatggactgcaggccagccccccggccacgctgaaggtggtggccatccggccggccatacagatccaccgcagcacagggttgcgactggcccaaggctctgccatgcccatcttgcccgccaacctgtcggtggagaccaatgccgtggggcaggatgtgagcgtgctgttccgcgtcactggggccctgcagtttggggagctgcagaagcagggggcaggtggggtggagggtgctgagtggtgggccacacaggcgttccaccagcgggatgtggagcagggccgcgtgaggtacctgagcactgacccacagcaccacgcttacgacaccgtggagaacctggccctggaggtgcaggtgggccaggagatcctgagcaatctgtccttcccagtgaccatccagagagccactgtgtggatgctgcggctggagccactgcacactcagaacacccagcaggagaccctcaccacagcccacctggaggccaccctggaggaggcaggcccaagccccccaaccttccattatgaggtggttcaggctcccaggaaaggcaaccttcaactacagggcacaaggctgtcagatggccagggcttcacccaggatgacatacaggctggccgggtgacctatggggccacagcacgtgcctcagaggcagtcgaggacaccttccgtttccgtgtcacagctccaccatatttctccccactctataccttccccatccacattggtggtgacccagatgcgcctgtcctcaccaatgtcctcctcgtggtgcctgagggtggtgagggtgtcctctctgctgaccacctctttgtcaagagtctcaacagtgccagctacctctatgaggtcatggagcggccccgccatgggaggttggcttggcgtgggacacaggacaagaccactatggtgacatccttcaccaatgaagacctgttgcgtggccggctggtctaccagcatgatgactccgagaccacagaagatgatatcccatttgttgctacccgccagggcgagagcagtggtgacatggcctgggaggaggtacggggtgtcttccgagtggccatccagcccgtgaatgaccacgcccctgtgcagaccatcagccggatcttccatgtggcccggggtgggcggcggctgctgactacagacgacgtggccttcagcgatgctgactcgggctttgctgacgcccagctggtgcttacccgcaaggacctcctctttggcagtatcgtggccgtagatgagcccacgcggcccatctaccgcttcacccaggaggacctcaggaagaggcgagtactgttcgtgcactcaggggctgaccgtggctggatccagctgcaggtgtccgacgggcaacaccaggccactgcgctgctggaggtgcaggcctcggaaccctacctccgtgtggccaacggctccagccttgtggtccctcaaggaggccagggcaccatcgacacggccgtgctccacctggacaccaacctcgacatccgcagtggggatgaggtccactaccacgtcacagctggccctcgctggggacagctagtccgggctggtcagccagccacagccttctcccagcaggacctgctggatggggccgttctctatagccacaatggcagcctcagcccccgcgacaccatggccttctccgtggaagcagggccagtgcacacggatgccaccctacaagtgaccattgccctagagggcccactggccccactgaagctggtccggcacaagaagatctacgtcttccagggggaggcagctgagatcagaaaggatcagctggaggcagcgcaggaggcagtgccgcccgcccaaattgtgttctcggtgaagaccccgccgcgggccggctacctggtgatgctgtcccgcggcgcctccgtggccgggccgcccagctgggaccccgtgcagagcttctcccaggaggcggtggacgccggcagggtcctgtacctccactcccgccccgaggcctggagtgactccttctccctagacgtgggctcaggcctgggtgcgcccctcgagggcgtccgcgtggagctggaggtgctgcccgccaccatcccactggaggcacagaacttcagcgtccccgagggcggcagccgcgtgctggcccccccgctgctccaggtcgccgggccctacttccctgcactgcccggcctcgaactgcgggtcctcgagcagcccctgcacggggccctgcggagagaggaggcccctcaagcggggaccctcagcgctttctcctggaaagaggtagaacagcagcagatccgctatgtgcacgacgggagtgagacgctgacagacagcttcaccctagtggctaacgcctccgagctggaccgccagagccaccctgtggccttcaccatcaccgtcctgcccgtcaatgaccaaccgcccatcctcaccgcaaacacaggcctaacgatgtgggagggggccaccgtgcccttccctccggaggccctgaggggtgcggacagcgactcgggcccggaggacctggtctacaccatcgagcggcccagcaacgggcaggtggtgctgcgggcggcgccaggcaccgaggtgcacagcttcacgcaggcccagctggacgacgggctcgtgctgttctcacacagaggagccctggacggaggcttccgcttcagcctgtccgacggcgagcacgcttcccccggacacttcttccgcgtgacggcccagaagcagctgctcctctccctggagggcagccggacgctgaccgtgtgcccagggtcggtccagccgctcagcagccagagcctgagagccagctccagtgccggcaccgatccgcagcacctgctctaccgggtggtgcagggcccccggctgggccgcctgctccgcgcccagcagggcggcaccggggaggtcctggtgaacttcacgcaagccgaggtatacgcgggggatgttgtgtatgagcacaagatgcctgctgagcccttctgggaggtccacgacgccctggagctccggctgtcctcgccccccgcccccgacgtggccgccaccctggaggtggccgtgtccttcgaggccgcctgcccgcagcgccccagccgcctctggaggaacgagggtctctgggtggccgagggccagcaggcggacatcaccagcgccgccctggacgcctccaacctgctggcgcgcgtccccgccgcgctgcgcgcccggcacgacgtgctgttccaggtgacgcggttcccggcgcggggccggctgctgctggcggggcgggcgctgcacgcgggccgggcgcacttcctgcagtcggagctggcggcggggctcctggcctacgcgcacggcggcgggggcgcgcagcccgacggcttcggcttccgcgcgcagctgcagggccccgcgggcgccgggccgggcgcgctccccgcgctccccgcgctccccgacgaggccttcgccgtgcgcgtgggggccgcggcgtccgagccgctgcgcctgccccgcggctcccgcgcgcccgtgtcccgcgcgcagctccgcgtgcagctcccgggcgccgcgcccgccgacgtgcagtacgaggtgcggcgcgcggcccccggcggcttcctgagcctcgcgggcgcgggcgcgggcccggtgcgccgcttctcgcaggccgacgtggacgcgggccgcctggccttcgtggccaacggcagcagcgtggcgggcgtgctgcagctgagcgcgtgggccggcgccagcccgcgcgtgcccgtggcgctggccgtggacgtgctgcccgccgccatcgaggtgcagctgcgcgcgcccctggaggtgccccaggcgctggggcgctgcgcgctcgggccgcggcagctgcgcgtcgtgtcggaccgcgccgagcccgaggccgcctaccgcgtgacccgggcgccgcgcttcgggcagctcctggtggcgggcaggccggccggcgccttcagccagcggcaggtggaccgcggcgacgtggagttcgccttcaccgacctgtcctccccgcgcgaccgcttcgccgtcctggcccacgcgcggggcgccaacgccacggccacggtggacgtcacggtcgcggcgctgctgcgggtcgggccccgggggccgtggccgcagggcgccaccctgcgcctggacccggccgtcctggacgccgccgagctggccaaccgcacgggcggggagccgcgcttccgcctgctggccgggccccggctgggccgcctggtgcgcgtggcccgcgcggggccggagcccgtggagcagttcacgcagcgggacctggagggcgggaggctggggctgcagctgggccgcgcccccggccccacgggcgacagcctcacgctggagctgtgggcgcccggcgtccccccggccgtggcctccctggacttccacaccgagccctacgacgcggcgcgcccctacggcgtggccctgctcagcctccccgaggaagccggggcacccgacagcggcgccccggccacgggccagccgggcgcgccaggccccagccccgggcccaccgcggccagcggcggcttcctgggcctcctggaggccaacatgttcagcatcatcatccccgtgtgcctggtcctcctgctcctggccctgctcctgccgctgctcttctacctgcgcaagcggaacaagacgggcaagcacgacgtccaggtgctgaccgccaagccccgcaacggcctggccggcgacacggagaccttccgcaaggtggagccgggccacgccatcccgctcacggccgtgcccggccaggggcccccgcccggcggccagcccgacccagagctgctgcagtactgtcggacacccaaccccgccctcaaaaacggccagtactgggtgtagtctaga

SEQ ID NO: 6 - DNA, 33 bp, artificial
  primer
ccggaattcgccatggccctcggtgctctgcag

SEQ ID NO: 7 - DNA, 28 bp, artificial
  primer
ggtctagacccacgtctagggagaagga

SEQ ID NO: 8 - DNA, 32 bp, artificial
  primer
ccggaattcgccgccgttctctatagccacaa

SEQ ID NO: 9 - DNA, 29 bp, artificial
  primer
ggtctagatcacacccagtactggccatt

SEQ ID NO: 10 - DNA, 8262 bp, artificial
  DoHu-CSPG4-1
gaattcatggccctcggtgctctgcagagctgctccatccgccactcagagtcccagggaccccttccttcaaagtgtcggggcctgggtgatgggctgggcctctggagaggtgggcaggggccatctgaggtgaccagagtgggccatttgggcagcctgcaggctccagccgagcgattccagcacccgctctccttgggcttcgacgggaacccactctccaatatcttctcagcatccacgctgtacgagcattggcgggacaggagggtcttctggtgctgccgcctggggccgggtggccaggtgggccaggctgctggcgaggttgcgggaggggagcgggtgcgcatggagctctcagaggaagtgcacaggctgcttctgggaactgggcgtgctgcccaggaggggcaggcaggggagggggttggaagagcccgccgcacaccctcactggcgcacacagatgtgggtgtgcgcacaagtatgaacaaccgcgagcaggtgcccaaggggccctcgggcctgggcctgctcctgctcccccagctcctggctccacccagctcccctcttgcctccaacatgccccctgccccaaccctgggcattcggggcgagcccgtgtcccacgggcggccgaggagctcggccatcaggcctttctgccaaagccgtgacctccgtcagcgtgatgcccgggaggtacacgtacgcacatgcgtgcacacgcgcgtgcaagtgttgctcagcagcctggcccagagcctagcaaggagagcgcccagcccctcagcagccatcccgggagaaacccccgactcaggattcacggcccccagcaccacggccaggggccttgggggcattggcaagagggcccaggaccccggagagttggtgctggagacagagacgtgggggcaggtggttcaggggttagagccagccagcgccttcacttccggcctggtacgggccctgaggccctatgacgatgtccctgcatccagcttcaacagaggggagtctacagacccaggctgggaaaagccagctgtagtcggctatggctccccagccatcgtgggaacaacagggccggatctgactgccccccagggacaatcagcagccttgcggcaggaagcaatacggcgtgatgcaggaagctggggcccatttggggtccagtacgtggtctccatctggcctcagcgccttcgctctttggtggactcgggctggcgactgcacccttactccaaagacagctgggagagaagtgagggggcagtgccagccaggaccgtgaagctgcgccagcacaaaacccgcatcgtccgcagcacctctcctcctccagcctccttctttggggagaaccacctgcaggtgccggtgaccacagctctgagcaacatagacctccggctacaattctccacgtcccagcccgaagccctgctcctcctggcagcaggccaggctgaccacctcctcctgcagctccactccggatacctgcaggtcagactcaccctgggccaggaggagctgaggctgcagaccccagctgagactccgctgagcgactccgccgtccactccgtggagctgactgtgtcagacagcgaggcctcgttgtccgtcgatgggctgctgaacgcctcagcccccgtcctgggagctcccctggaggtcccctatgggatcttcctggggggcactgggagcctgagcctgtcctacctgatgggagccagccggcccctgaggggctgcctgcacgccgccaccgtcaacggccgcaacctcctccgaccactgacccctgacgtgcacgagggctgcgctgaagagttttctgctgatgacagcgtggctctgggcttctctgggccccactcgctggctgccttccctgcctggaacactcgggaggagggcaccctggcgttcatactcaccactcggagccgacaggcgcccctggctttccaggcgggcggccggcacggggatttcatctacgtggacatatttgagggccacctgcgggctgtggtggagaagggccagggcaccgtgttgctccacaacagcgtgcccgtggctgacgggctaccccatgaggtcagtgtccacgtggatgctcaccagctggaaatctccgtggaccagtaccccacacggacttccaaccgtgggatcctcagctacctggaaccccgcggcagtctcctcctgggggggctggacacagaggcctcccgccacctccaggaacaccgcctgggcctggcctcgggggccgtcaacgtctccctcctgggctgcatggaggatctcagcatcaacggccagaggcaggggctccgggaagcctcgctgactcgcagcatggtggccggctgcagcctggaggaagacgagtacgaggaggacacctacggcacctatgaagctctctccaccctggcaccggaggcctggtccgccgtggagctgcccgagccctgcgtgcccgaaccggggctgcctcccgtctttgccaacttcacccaactgctgactgtcagcccgctggtggtggccgaggggggcacagcctggcttgagtggcggcacctgcagcccacgctggacctgagcgaggccgagctgcgtaaatcccaggtgctgttcagcgtgagccgtggggcccgccacggggagctcgagctggacgtcccgggagcccaggcacggaaaatgttcaccctcctggacgtggtgaaccgcaaggcccgcttcgtccacgatggctcggaggagacctccgaccagctgatgctggaggtgtccgtgaccgccaggggccctgtgccctcctgcctccggaggggccagacttacatcctgcccatccagataaacccggtcaacgacccaccccaaatcatcttcccccacggcagcctcatggtgatcctggaacacacacagaagcccctggggcccgaggtcttccaggcctacgacccagactctgcctgcgagggcctcaccttccagctccttggcaccgccccgggcctgccggtggagcgccaggagcagcccggggagccagccaccgagttctcctgccgggagctggaggcgggcggcctggtctacgtgcaccggagcgggcccgcccaggacctgacgttccgcgtcagcgacgggctgcaggccagcgctccggccacgctgcaggtggtggcggtccggcccagcatccgggtccgccacaacacggggctgcgcctggcccagggctccgccgccccggtgctgcccgccaatctgtcggtggagaccaacgcggtggggcaggatgtgagcgtgctgttccgggtcgccgcggccctgcggttcggggagctgcagaagcagggcgcggggggcgccgagggcgcggagtggcgcccggtgcaggccttccagcagcgggacgtggagcagggccgcgtgaggtacctgagcaccgacccgcagcaccgcacggaggacgccgtggagcgcgtggccctggaggttcaggtgggccaggagaccctgagcaatctgtccttcctggtgacgatccagagagccaccgtgcggctgctgcggctcgagcccctgcgcacccacaccacgcggcaggaggcgctcaccggcgcgcacctggaggccgctctggaggagggggcgggccccagccccaccaccttccactacgagctggttcaggcccccaggaagggtaacctcaggctgcagggcgcccggctgtccgaggggcagggcttcacccaggatgacctgcaggccggccgggtgacctacggggccacggcgcgcacctcggagaccgtggaggacgccttccgtttccgcgtcacggctccgccacatttctccccgctctacaccttccccatccacatcgggggtgaccccgacgcccccgtcctcaccaacgtcctcctctccgtgcccgagggaggcgagggcgtcctctccgcggaacacctgttcgtcaagagcctcaacagcgccagctacctctatgaggtcatggagcggccccgccacgggcggctggtctggaggggggcgcaggacgaggccaccgcggtgacgtccttcaccaacgaggacctgctgcagggccggctggtctaccagcatgacaactccgagaccacggaagacgacatccccttcgtggcaacccgccagagtgagggcagcggcggcctggcctgggaggaggtccggggcgtcttccgcgtggccatccagcccgtgaacgaccacgctcccgtgcagaccgtcagccgcgtcttccacgtggcccggggcgggcggcggctgctgacgaccgacgacgtggccttcagtgacgccgactccggcttcgccgacgcgcagctggtgctgacccgcaaggaccttctcttcggcagcatcgtggccgcggacgagcccacgcggcccatctaccgcttctcccaggaggacctccggaagaggcgcgtcctgttcgtgcactccggggccgaccgcggctggatccagctgcaggtgtccgacgggcggcaccaggccaccgcgctgcttgaagtgcaggcatccgagccctatctccgcgtggccaatggctccagcctcgtggtccctcaggggggccagggcaccatcgacacagccgtgctccgcctggacaccaacctagacattcgcagcggggatgaggtccgctaccgtgtcacagccggcccgcactgggggcagctgctccgggccggccagccggccacagccttctcccaacaggacctgctggacggggccgtcctctacagccacaacggcagcctgagcccgcaggacaccctggccttctccgtggaggcagggcctgtgctcacggatgccaccctgcaggtgaccattgccttggaggggccattggccccactgcatctggtccagaacaagaagatctacgtcttccagggagaggcagctgagatcagaagggaccagctggaggcagcccaggaggcagtgccacctgcagacatcgtattctcagtgaagagcccaccgagtgccggctacctggtgatggtgtcgcgtggcgccttggcagatgagccacccagcctggaccctgtgcagagcttctcccaggaggcagtggacacaggcagggtcctgtacctgcactcccgccctgaggcctggagcgatgccttctcgctggatgtggcctcaggcctgggtgctcccctcgagggcgtccttgtggagctggaggtgctgcccgctgccatcccactagaggcgcaaaacttcagcgtccctgagggtggcagcctcaccctggcccctccactgctccgtgtctccgggccctacttccccactctcctgggcctcagcctgcaggtgctggagccaccccagcatggagccctgcagaaggaggacggacctcaagccaggaccctcagcgccttctcctggagaatggtggaagagcagctgatccgctacgtgcatgacgggagcgagacactgacagacagttttgtcctgatggctaatgcctccgagatggatcgccagagccatcctgtggccttcactgtcactgtcctgcctgtcaatgaccaaccccccatcctcactacaaacacaggcctgcagatgtgggagggggccactgcgcccatccctgcggaggctctgaggagcacggacggcgactctgggtctgaggatctggtctacaccatcgagcagcccagcaacgggcgggtagtgctgcggggggcgccgggcactgaggtgcgcagcttcacgcaggcccagctggacggcgggctcgtgctgttctcacacagaggaaccctggatggaggcttccgcttccgcctctctgacggcgagcacacttcccccggacacttcttccgagtgacggcccagaagcaagtgctcctctcgctgaagggcagccagacactgactgtctgcccagggtccgtccagccactcagcagtcagaccctcagggccagctccagcgcaggcactgacccccagctcctgctctaccgtgtggtgcggggcccccagctaggccggctgttccacgcccagcaggacagcacaggggaggccctggtgaacttcactcaggcagaggtctacgctgggaatattctgtatgagcatgagatgccccccgagcccttttgggaggcccatgataccctagagctccagctgtcctcgccgcctgcccgggacgtggccgccacccttgctgtggctgtgtcttttgaggctgcctgtccccagcgccccagccacctctggaagaacaaaggtctctgggtccccgagggccagcgggccaggatcaccgtggctgctctggatgcctccaatctcttggccagcgttccatcaccccagcgctcagagcatgatgtgctcttccaggtcacacagttccccagccggggccagctgttggtgtccgaggagcccctccatgctgggcagccccacttcctgcagtcccagctggctgcagggcagctagtgtatgcccacggcggtgggggcacccagcaggatggcttccactttcgtgcccacctccaggggccagcaggggcctccgtggctggaccccaaacctcagaggcctttgccatcacggtgagggatgtaaatgagcggccccctcagccacaggcctctgtcccactccggctcacccgaggctctcgtgcccccatctcccgggcccagctgagtgtggtggacccagactcagctcctggggagattgagtacgaggtccagcgggcaccccacaacggcttcctcagcctggtgggtggtggcctggggcccgtgacccgcttcacgcaagccgatgtggattcagggcggctggccttcgtggccaacgggagcagcgtggcaggcatcttccagctgagcatgtctgatggggccagcccacccctgcccatgtccctggctgtggacatcctaccatccgccatcgaggtgcagctgcgggcacccctggaggtgccccaagctttggggcgctcctcactgagccagcagcagctccgggtggtttcagatcgggaggagccagaggcagcataccgcctcatccagggaccccagtatgggcatctcctggtgggcgggcggcccacctcggccttcagccaattccagatagaccagggcgaggtggtctttgccttcaccaacttctcctcctctcatgaccacttcagagtcctggcactggctaggggtgtcaatgcatcagccgtagtgaacgtcactgtgagggctctgctgcatgtgtgggcaggtgggccatggccccagggtgccaccctgcgcctggaccccaccgtcctagatgctggcgagctggccaaccgcacaggcagtgtgccgcgcttccgcctcctggagggaccccggcatggccgcgtggtccgcgtgccccgagccaggacggagcccgggggcagccagctggtggagcagttcactcagcaggaccttgaggacgggaggctggggctggaggtgggcaggccagaggggagggcccccggccccgcaggtgacagtctcactctggagctgtgggcacagggcgtcccgcctgctgtggcctccctggactttgccactgagccttacaatgctgcccggccctacagcgtggccctgctcagtgtccccgaggccgcccggacggaagcagggaagccagagagcagcacccccacaggcgagccaggccccatggcatccagccctgagcccgctgtggccaagggaggcttcctgagcttccttgaggccaacatgttcagcgtcatcatccccatgtgcctggtacttctgctcctggcgctcatcctgcccctgctcttctacctccgaaaacgcaacaagacgggcaagcatgacgtccaggtcctgactgccaagccccgcaacggcctggctggtgacaccgagacctttcgcaaggtggagccaggccaggccatcccgctcacagctgtgcctggccaggggccccctccaggaggccagcctgacccagagctgctgcagttctgccggacacccaaccctgcccttaagaatggccagtactgggtgtgatctaga

SEQ ID NO: 11 - DNA, 1920 bp, artificial
  HUMAN D1
atgcagtccgggccgcggcccccacttccagcccccggcctggccttggctttgaccctgactatgttggccagacttgcatccgcggcttccttcttcggtgagaaccacctggaggtgcctgtggccacggctctgaccgacatagacctgcagctgcagttctccacgtcccagcccgaagccctccttctcctggcagcaggcccagctgaccacctcctgctgcagctctactctggacgcctgcaggtcagacttgttctgggccaggaggagctgaggctgcagactccagcagagacgctgctgagtgactccatcccccacactgtggtgctgactgtcgtagagggctgggccacgttgtcagtcgatgggtttctgaacgcctcctcagcagtcccaggagcccccctagaggtcccctatgggctctttgttgggggcactgggacccttggcctgccctacctgaggggaaccagccgacccctgaggggttgcctccatgcagccaccctcaatggccgcagcctcctccggcctctgacccccgatgtgcatgagggctgtgctgaagagttttctgccagtgatgatgtggccctgggcttctctgggccccactctctggctgccttccctgcctggggcactcaggacgaaggaaccctagagtttacactcaccacacagagccggcaggcacccttggccttccaggcagggggccggcgtggggacttcatctatgtggacatatttgagggccacctgcgggccgtggtggagaagggccagggtaccgtattgctccacaacagtgtgcctgtggccgatgggcagccccatgaggtcagtgtccacatcaatgctcaccggctggaaatctccgtggaccagtaccctacgcatacttcgaaccgaggagtcctcagctacctggagccacggggcagtctccttctcggggggctggatgcagaggcctctcgtcacctccaggaacaccgcctgggcctgacaccagaggccaccaatgcctccctgctgggctgcatggaagacctcagtgtcaatggccagaggcgggggctgcgggaagctttgctgacgcgcaacatggcagccggctgcaggctggaggaggaggagtatgaggacgatgcctatggacattatgaagctttctccaccctggcccctgaggcttggccagccatggagctgcctgagccatgcgtgcctgagccagggctgcctcctgtctttgccaatttcacccagctgctgactatcagcccactggtggtggccgaggggggcacagcctggcttgagtggaggcatgtgcagcccacgctggacctgatggaggctgagctgcgcaaatcccaggtgctgttcagcgtgacccgaggggcacgccatggcgagctcgagctggacatcccgggagcccaggcacgaaaaatgttcaccctcctggacgtggtgaaccgcaaggcccgcttcatccacgatggctctgaggacacctccgaccagctggtgctggaggtgtcggtgacggctcgggtgcccatgccctcatgccttcggaggggccaaacatacctcctgcccatccaggtcaaccctgtcaatgacccaccccacatcatcttcccacatggcagcctcatggtgatcctggaacacacgcagaagccgctggggcctgaggttttccaggcctatgacccggactctgcctgtgagggcctcaccttccaggtccttggcacctcctctggcctccccgtggagcgccgagaccagcctggggagccggcgaccgagttctcctgccgggagttggaggccggcagcctagtctatgtccaccgcggtggtcctgcacaggacttgacgttc

SEQ ID NO: 12 - DNA, 4767 bp, artificial
  Human D1+D2
atgcagtccgggccgcggcccccacttccagcccccggcctggccttggctttgaccctgactatgttggccagacttgcatccgcggcttccttcttcggtgagaaccacctggaggtgcctgtggccacggctctgaccgacatagacctgcagctgcagttctccacgtcccagcccgaagccctccttctcctggcagcaggcccagctgaccacctcctgctgcagctctactctggacgcctgcaggtcagacttgttctgggccaggaggagctgaggctgcagactccagcagagacgctgctgagtgactccatcccccacactgtggtgctgactgtcgtagagggctgggccacgttgtcagtcgatgggtttctgaacgcctcctcagcagtcccaggagcccccctagaggtcccctatgggctctttgttgggggcactgggacccttggcctgccctacctgaggggaaccagccgacccctgaggggttgcctccatgcagccaccctcaatggccgcagcctcctccggcctctgacccccgatgtgcatgagggctgtgctgaagagttttctgccagtgatgatgtggccctgggcttctctgggccccactctctggctgccttccctgcctggggcactcaggacgaaggaaccctagagtttacactcaccacacagagccggcaggcacccttggccttccaggcagggggccggcgtggggacttcatctatgtggacatatttgagggccacctgcgggccgtggtggagaagggccagggtaccgtattgctccacaacagtgtgcctgtggccgatgggcagccccatgaggtcagtgtccacatcaatgctcaccggctggaaatctccgtggaccagtaccctacgcatacttcgaaccgaggagtcctcagctacctggagccacggggcagtctccttctcggggggctggatgcagaggcctctcgtcacctccaggaacaccgcctgggcctgacaccagaggccaccaatgcctccctgctgggctgcatggaagacctcagtgtcaatggccagaggcgggggctgcgggaagctttgctgacgcgcaacatggcagccggctgcaggctggaggaggaggagtatgaggacgatgcctatggacattatgaagctttctccaccctggcccctgaggcttggccagccatggagctgcctgagccatgcgtgcctgagccagggctgcctcctgtctttgccaatttcacccagctgctgactatcagcccactggtggtggccgaggggggcacagcctggcttgagtggaggcatgtgcagcccacgctggacctgatggaggctgagctgcgcaaatcccaggtgctgttcagcgtgacccgaggggcacgccatggcgagctcgagctggacatcccgggagcccaggcacgaaaaatgttcaccctcctggacgtggtgaaccgcaaggcccgcttcatccacgatggctctgaggacacctccgaccagctggtgctggaggtgtcggtgacggctcgggtgcccatgccctcatgccttcggaggggccaaacatacctcctgcccatccaggtcaaccctgtcaatgacccaccccacatcatcttcccacatggcagcctcatggtgatcctggaacacacgcagaagccgctggggcctgaggttttccaggcctatgacccggactctgcctgtgagggcctcaccttccaggtccttggcacctcctctggcctccccgtggagcgccgagaccagcctggggagccggcgaccgagttctcctgccgggagttggaggccggcagcctagtctatgtccaccgcggtggtcctgcacaggacttgacgttccgggtcagcgatggactgcaggccagccccccggccacgctgaaggtggtggccatccggccggccatacagatccaccgcagcacagggttgcgactggcccaaggctctgccatgcccatcttgcccgccaacctgtcggtggagaccaatgccgtggggcaggatgtgagcgtgctgttccgcgtcactggggccctgcagtttggggagctgcagaagcagggggcaggtggggtggagggtgctgagtggtgggccacacaggcgttccaccagcgggatgtggagcagggccgcgtgaggtacctgagcactgacccacagcaccacgcttacgacaccgtggagaacctggccctggaggtgcaggtgggccaggagatcctgagcaatctgtccttcccagtgaccatccagagagccactgtgtggatgctgcggctggagccactgcacactcagaacacccagcaggagaccctcaccacagcccacctggaggccaccctggaggaggcaggcccaagccccccaaccttccattatgaggtggttcaggctcccaggaaaggcaaccttcaactacagggcacaaggctgtcagatggccagggcttcacccaggatgacatacaggctggccgggtgacctatggggccacagcacgtgcctcagaggcagtcgaggacaccttccgtttccgtgtcacagctccaccatatttctccccactctataccttccccatccacattggtggtgacccagatgcgcctgtcctcaccaatgtcctcctcgtggtgcctgagggtggtgagggtgtcctctctgctgaccacctctttgtcaagagtctcaacagtgccagctacctctatgaggtcatggagcggccccgccatgggaggttggcttggcgtgggacacaggacaagaccactatggtgacatccttcaccaatgaagacctgttgcgtggccggctggtctaccagcatgatgactccgagaccacagaagatgatatcccatttgttgctacccgccagggcgagagcagtggtgacatggcctgggaggaggtacggggtgtcttccgagtggccatccagcccgtgaatgaccacgcccctgtgcagaccatcagccggatcttccatgtggcccggggtgggcggcggctgctgactacagacgacgtggccttcagcgatgctgactcgggctttgctgacgcccagctggtgcttacccgcaaggacctcctctttggcagtatcgtggccgtagatgagcccacgcggcccatctaccgcttcacccaggaggacctcaggaagaggcgagtactgttcgtgcactcaggggctgaccgtggctggatccagctgcaggtgtccgacgggcaacaccaggccactgcgctgctggaggtgcaggcctcggaaccctacctccgtgtggccaacggctccagccttgtggtccctcaaggaggccagggcaccatcgacacggccgtgctccacctggacaccaacctcgacatccgcagtggggatgaggtccactaccacgtcacagctggccctcgctggggacagctagtccgggctggtcagccagccacagccttctcccagcaggacctgctggatggggccgttctctatagccacaatggcagcctcagcccccgcgacaccatggccttctccgtggaagcagggccagtgcacacggatgccaccctacaagtgaccattgccctagagggcccactggccccactgaagctggtccggcacaagaagatctacgtcttccagggagaggcagctgagatcagaagggaccagctggaggcagcccaggaggcagtgccacctgcagacatcgtattctcagtgaagagcccaccgagtgccggctacctggtgatggtgtcgcgtggcgccttggcagatgagccacccagcctggaccctgtgcagagcttctcccaggaggcagtggacacaggcagggtcctgtacctgcactcccgccctgaggcctggagcgatgccttctcgctggatgtggcctcaggcctgggtgctcccctcgagggcgtccttgtggagctggaggtgctgcccgctgccatcccactagaggcgcaaaacttcagcgtccctgagggtggcagcctcaccctggcccctccactgctccgtgtctccgggccctacttccccactctcctgggcctcagcctgcaggtgctggagccaccccagcatggagccctgcagaaggaggacggacctcaagccaggaccctcagcgccttctcctggagaatggtggaagagcagctgatccgctacgtgcatgacgggagcgagacactgacagacagttttgtcctgatggctaatgcctccgagatggatcgccagagccatcctgtggccttcactgtcactgtcctgcctgtcaatgaccaaccccccatcctcactacaaacacaggcctgcagatgtgggagggggccactgcgcccatccctgcggaggctctgaggagcacggacggcgactctgggtctgaggatctggtctacaccatcgagcagcccagcaacgggcgggtagtgctgcggggggcgccgggcactgaggtgcgcagcttcacgcaggcccagctggacggcgggctcgtgctgttctcacacagaggaaccctggatggaggcttccgcttccgcctctctgacggcgagcacacttcccccggacacttcttccgagtgacggcccagaagcaagtgctcctctcgctgaagggcagccagaca

SEQ ID NO: 13 - DNA, 1965 bp, artificial
  Dog D1
atgggctccccgcgctccggctccgcccggccccgccgacctgccgcgatgcggggtcagccgcccgcgcccccgggccccgcgctgcccctggccttggccttggctctgtgggcctgcgccgcctccgcggcctccttctttggggagaaccacctgcaggtgccggtgaccacagctctgagcaacatagacctccggctacaattctccacgtcccagcccgaagccctgctcctcctggcagcaggccaggctgaccacctcctcctgcagctccactccggatacctgcaggtcagactcaccctgggccaggaggagctgaggctgcagaccccagctgagactccgctgagcgactccgccgtccactccgtggagctgactgtgtcagacagcgaggcctcgttgtccgtcgatgggctgctgaacgcctcagcccccgtcctgggagctcccctggaggtcccctatgggatcttcctggggggcactgggagcctgagcctgtcctacctgatgggagccagccggcccctgaggggctgcctgcacgccgccaccgtcaacggccgcaacctcctccgaccactgacccctgacgtgcacgagggctgcgctgaagagttttctgctgatgacagcgtggctctgggcttctctgggccccactcgctggctgccttccctgcctggaacactcgggaggagggcaccctggcgttcatactcaccactcggagccgacaggcgcccctggctttccaggcgggcggccggcacggggatttcatctacgtggacatatttgagggccacctgcgggctgtggtggagaagggccagggcaccgtgttgctccacaacagcgtgcccgtggctgacgggctaccccatgaggtcagtgtccacgtggatgctcaccagctggaaatctccgtggaccagtaccccacacggacttccaaccgtgggatcctcagctacctggaaccccgcggcagtctcctcctgggggggctggacacagaggcctcccgccacctccaggaacaccgcctgggcctggcctcgggggccgtcaacgtctccctcctgggctgcatggaggatctcagcatcaacggccagaggcaggggctccgggaagcctcgctgactcgcagcatggtggccggctgcagcctggaggaagacgagtacgaggaggacacctacggcacctatgaagctctctccaccctggcaccggaggcctggtccgccgtggagctgcccgagccctgcgtgcccgaaccggggctgcctcccgtctttgccaacttcacccaactgctgactgtcagcccgctggtggtggccgaggggggcacagcctggcttgagtggcggcacctgcagcccacgctggacctgagcgaggccgagctgcgtaaatcccaggtgctgttcagcgtgagccgtggggcccgccacggggagctcgagctggacgtcccgggagcccaggcacggaaaatgttcaccctcctggacgtggtgaaccgcaaggcccgcttcgtccacgatggctcggaggagacctccgaccagctgatgctggaggtgtccgtgaccgccaggggccctgtgccctcctgcctccggaggggccagacttacatcctgcccatccagataaacccggtcaacgacccaccccaaatcatcttcccccacggcagcctcatggtgatcctggaacacacacagaagcccctggggcccgaggtcttccaggcctacgacccagactctgcctgcgagggcctcaccttccagctccttggcaccgccccgggcctgccggtggagcgccaggagcagcccggggagccagccaccgagttctcctgccgggagctggaggcgggcggcctggtctacgtgcaccggagcgggcccgcccaggacctgacgttc

SEQ ID NO: 14 - DNA, 4815 bp, artificial
  Dog D1+D2
atgggctccccgcgctccggctccgcccggccccgccgacctgccgcgatgcggggtcagccgcccgcgcccccgggccccgcgctgcccctggccttggccttggctctgtgggcctgcgccgcctccgcggcctccttctttggggagaaccacctgcaggtgccggtgaccacagctctgagcaacatagacctccggctacaattctccacgtcccagcccgaagccctgctcctcctggcagcaggccaggctgaccacctcctcctgcagctccactccggatacctgcaggtcagactcaccctgggccaggaggagctgaggctgcagaccccagctgagactccgctgagcgactccgccgtccactccgtggagctgactgtgtcagacagcgaggcctcgttgtccgtcgatgggctgctgaacgcctcagcccccgtcctgggagctcccctggaggtcccctatgggatcttcctggggggcactgggagcctgagcctgtcctacctgatgggagccagccggcccctgaggggctgcctgcacgccgccaccgtcaacggccgcaacctcctccgaccactgacccctgacgtgcacgagggctgcgctgaagagttttctgctgatgacagcgtggctctgggcttctctgggccccactcgctggctgccttccctgcctggaacactcgggaggagggcaccctggcgttcatactcaccactcggagccgacaggcgcccctggctttccaggcgggcggccggcacggggatttcatctacgtggacatatttgagggccacctgcgggctgtggtggagaagggccagggcaccgtgttgctccacaacagcgtgcccgtggctgacgggctaccccatgaggtcagtgtccacgtggatgctcaccagctggaaatctccgtggaccagtaccccacacggacttccaaccgtgggatcctcagctacctggaaccccgcggcagtctcctcctgggggggctggacacagaggcctcccgccacctccaggaacaccgcctgggcctggcctcgggggccgtcaacgtctccctcctgggctgcatggaggatctcagcatcaacggccagaggcaggggctccgggaagcctcgctgactcgcagcatggtggccggctgcagcctggaggaagacgagtacgaggaggacacctacggcacctatgaagctctctccaccctggcaccggaggcctggtccgccgtggagctgcccgagccctgcgtgcccgaaccggggctgcctcccgtctttgccaacttcacccaactgctgactgtcagcccgctggtggtggccgaggggggcacagcctggcttgagtggcggcacctgcagcccacgctggacctgagcgaggccgagctgcgtaaatcccaggtgctgttcagcgtgagccgtggggcccgccacggggagctcgagctggacgtcccgggagcccaggcacggaaaatgttcaccctcctggacgtggtgaaccgcaaggcccgcttcgtccacgatggctcggaggagacctccgaccagctgatgctggaggtgtccgtgaccgccaggggccctgtgccctcctgcctccggaggggccagacttacatcctgcccatccagataaacccggtcaacgacccaccccaaatcatcttcccccacggcagcctcatggtgatcctggaacacacacagaagcccctggggcccgaggtcttccaggcctacgacccagactctgcctgcgagggcctcaccttccagctccttggcaccgccccgggcctgccggtggagcgccaggagcagcccggggagccagccaccgagttctcctgccgggagctggaggcgggcggcctggtctacgtgcaccggagcgggcccgcccaggacctgacgttccgcgtcagcgacgggctgcaggccagcgctccggccacgctgcaggtggtggcggtccggcccagcatccgggtccgccacaacacggggctgcgcctggcccagggctccgccgccccggtgctgcccgccaatctgtcggtggagaccaacgcggtggggcaggatgtgagcgtgctgttccgggtcgccgcggccctgcggttcggggagctgcagaagcagggcgcggggggcgccgagggcgcggagtggcgcccggtgcaggccttccagcagcgggacgtggagcagggccgcgtgaggtacctgagcaccgacccgcagcaccgcacggaggacgccgtggagcgcgtggccctggaggttcaggtgggccaggagaccctgagcaatctgtccttcctggtgacgatccagagagccaccgtgcggctgctgcggctcgagcccctgcgcacccacaccacgcggcaggaggcgctcaccggcgcgcacctggaggccgctctggaggagggggcgggccccagccccaccaccttccactacgagctggttcaggcccccaggaagggtaacctcaggctgcagggcgcccggctgtccgaggggcagggcttcacccaggatgacctgcaggccggccgggtgacctacggggccacggcgcgcacctcggagaccgtggaggacgccttccgtttccgcgtcacggctccgccacatttctccccgctctacaccttccccatccacatcgggggtgaccccgacgcccccgtcctcaccaacgtcctcctctccgtgcccgagggaggcgagggcgtcctctccgcggaacacctgttcgtcaagagcctcaacagcgccagctacctctatgaggtcatggagcggccccgccacgggcggctggtctggaggggggcgcaggacgaggccaccgcggtgacgtccttcaccaacgaggacctgctgcagggccggctggtctaccagcatgacaactccgagaccacggaagacgacatccccttcgtggcaacccgccagagtgagggcagcggcggcctggcctgggaggaggtccggggcgtcttccgcgtggccatccagcccgtgaacgaccacgctcccgtgcagaccgtcagccgcgtcttccacgtggcccggggcgggcggcggctgctgacgaccgacgacgtggccttcagtgacgccgactccggcttcgccgacgcgcagctggtgctgacccgcaaggaccttctcttcggcagcatcgtggccgcggacgagcccacgcggcccatctaccgcttctcccaggaggacctccggaagaggcgcgtcctgttcgtgcactccggggccgaccgcggctggatccagctgcaggtgtccgacgggcggcaccaggccaccgcgctgcttgaagtgcaggcatccgagccctatctccgcgtggccaatggctccagcctcgtggtccctcaggggggccagggcaccatcgacacagccgtgctccgcctggacaccaacctagacattcgcagcggggatgaggtccgctaccgtgtcacagccggcccgcactgggggcagctgctccgggccggccagccggccacagccttctcccaacaggacctgctggacggggccgtcctctacagccacaacggcagcctgagcccgcaggacaccctggccttctccgtggaggcagggcctgtgctcacggatgccaccctgcaggtgaccattgccttggaggggccattggccccactgcatctggtccagaacaagaagatctacgtcttccagggggaggcagctgagatcagaaaggatcagctggaggcagcgcaggaggcagtgccgcccgcccaaattgtgttctcggtgaagaccccgccgcgggccggctacctggtgatgctgtcccgcggcgcctccgtggccgggccgcccagctgggaccccgtgcagagcttctcccaggaggcggtggacgccggcagggtcctgtacctccactcccgccccgaggcctggagtgactccttctccctagacgtgggctcaggcctgggtgcgcccctcgagggcgtccgcgtggagctggaggtgctgcccgccaccatcccactggaggcacagaacttcagcgtccccgagggcggcagccgcgtgctggcccccccgctgctccaggtcgccgggccctacttccctgcactgcccggcctcgaactgcgggtcctcgagcagcccctgcacggggccctgcggagagaggaggcccctcaagcggggaccctcagcgctttctcctggaaagaggtagaacagcagcagatccgctatgtgcacgacgggagtgagacgctgacagacagcttcaccctagtggctaacgcctccgagctggaccgccagagccaccctgtggccttcaccatcaccgtcctgcccgtcaatgaccaaccgcccatcctcaccgcaaacacaggcctaacgatgtgggagggggccaccgtgcccttccctccggaggccctgaggggtgcggacagcgactcgggcccggaggacctggtctacaccatcgagcggcccagcaacgggcaggtggtgctgcgggcggcgccaggcaccgaggtgcacagcttcacgcaggcccagctggacgacgggctcgtgctgttctcacacagaggagccctggacggaggcttccgcttcagcctgtccgacggcgagcacgcttcccccggacacttcttccgcgtgacggcccagaagcagctgctcctctccctggagggcagccggacg

SEQ ID NO: 15 - DNA, 3737 bp, artificial
  HuDo Hu
atgcagtccgggccgcggcccccacttccagcccccggcctggccttggctttgaccctgactatgttggccagacttgcatccgcggcttccttcttcggtgagaaccacctggaggtgcctgtggccacggctctgaccgacatagacctgcagctgcagttctccacgtcccagcccgaagccctccttctcctggcagcaggcccagctgaccacctcctgctgcagctctactctggacgcctgcaggtcagacttgttctgggccaggaggagctgaggctgcagactccagcagagacgctgctgagtgactccatcccccacactgtggtgctgactgtcgtagagggctgggccacgttgtcagtcgatgggtttctgaacgcctcctcagcagtcccaggagcccccctagaggtcccctatgggctctttgttgggggcactgggacccttggcctgccctacctgaggggaaccagccgacccctgaggggttgcctccatgcagccaccctcaatggccgcagcctcctccggcctctgacccccgatgtgcatgagggctgtgctgaagagttttctgccagtgatgatgtggccctgggcttctctgggccccactctctggctgccttccctgcctggggcactcaggacgaaggaaccctagagtttacactcaccacacagagccggcaggcacccttggccttccaggcagggggccggcgtggggacttcatctatgtggacatatttgagggccacctgcgggccgtggtggagaagggccagggtaccgtattgctccacaacagtgtgcctgtggccgatgggcagccccatgaggtcagtgtccacatcaatgctcaccggctggaaatctccgtggaccagtaccctacgcatacttcgaaccgaggagtcctcagctacctggagccacggggcagtctccttctcggggggctggatgcagaggcctctcgtcacctccaggaacaccgcctgggcctgacaccagaggccaccaatgcctccctgctgggctgcatggaagacctcagtgtcaatggccagaggcgggggctgcgggaagctttgctgacgcgcaacatggcagccggctgcaggctggaggaggaggagtatgaggacgatgcctatggacattatgaagctttctccaccctggcccctgaggcttggccagccatggagctgcctgagccatgcgtgcctgagccagggctgcctcctgtctttgccaatttcacccagctgctgactatcagcccactggtggtggccgaggggggcacagcctggcttgagtggaggcatgtgcagcccacgctggacctgatggaggctgagctgcgcaaatcccaggtgctgttcagcgtgacccgaggggcacgccatggcgagctcgagctggacatcccgggagcccaggcacgaaaaatgttcaccctcctggacgtggtgaaccgcaaggcccgcttcatccacgatggctctgaggacacctccgaccagctggtgctggaggtgtcggtgacggctcgggtgcccatgccctcatgccttcggaggggccaaacatacctcctgcccatccaggtcaaccctgtcaatgacccaccccacatcatcttcccacatggcagcctcatggtgatcctggaacacacgcagaagccgctggggcctgaggttttccaggcctatgacccggactctgcctgtgagggcctcaccttccaggtccttggcacctcctctggcctccccgtggagcgccgagaccagcctggggagccggcgaccgagttctcctgccgggagttggaggccggcagcctagtctatgtccaccgcggtggtcctgcacaggacttgacgttccgggtcagcgatggactgcaggccagccccccggccacgctgaaggtggtggccatccggccggccatacagatccaccgcagcacagggttgcgactggcccaaggctctgccatgcccatcttgcccgccaacctgtcggtggagaccaatgccgtggggcaggatgtgagcgtgctgttccgcgtcactggggccctgcagtttggggagctgcagaagcagggggcaggtggggtggagggtgctgagtggtgggccacacaggcgttccaccagcgggatgtggagcagggccgcgtgaggtacctgagcactgacccacagcaccacgcttacgacaccgtggagaacctggccctggaggtgcaggtgggccaggagatcctgagcaatctgtccttcccagtgaccatccagagagccactgtgtggatgctgcggctggagccactgcacactcagaacacccagcaggagaccctcaccacagcccacctggaggccaccctggaggaggcaggcccaagccccccaaccttccattatgaggtggttcaggctcccaggaaaggcaaccttcaactacagggcacaaggctgtcagatggccagggcttcacccaggatgacatacaggctggccgggtgacctatggggccacagcacgtgcctcagaggcagtcgaggacaccttccgtttccgtgtcacagctccaccatatttctccccactctataccttccccatccacattggtggtgacccagatgcgcctgtcctcaccaatgtcctcctcgtggtgcctgagggtggtgagggtgtcctctctgctgaccacctctttgtcaagagtctcaacagtgccagctacctctatgaggtcatggagcggccccgccatgggaggttggcttggcgtgggacacaggacaagaccactatggtgacatccttcaccaatgaagacctgttgcgtggccggctggtctaccagcatgatgactccgagaccacagaagatgatatcccatttgttgctacccgccagggcgagagcagtggtgacatggcctgggaggaggtacggggtgtcttccgagtggccatccagcccgtgaatgaccacgcccctgtgcagaccatcagccggatcttccatgtggcccggggtgggcggcggctgctgactacagacgacgtggccttcagcgatgctgactcgggctttgctgacgcccagctggtgcttacccgcaaggacctcctctttggcagtatcgtggccgtagatgagcccacgcggcccatctaccgcttcacccaggaggacctcaggaagaggcgagtactgttcgtgcactcaggggctgaccgtggctggatccagctgcaggtgtccgacgggcaacaccaggccactgcgctgctggaggtgcaggcctcggaaccctacctccgtgtggccaacggctccagccttgtggtccctcaaggaggccagggcaccatcgacacggccgtgctccacctggacaccaacctcgacatccgcagtggggatgaggtccactaccacgtcacagctggccctcgctggggacagctagtccgggctggtcagccagccacagccttctcccagcaggacctgctggatggggccgttctctatagccacaatggcagcctcagcccccgcgacaccatggccttctccgtggaagcagggccagtgcacacggatgccaccctacaagtgaccattgccctagagggcccactggccccactgaagctggtccggcacaagaa

SEQ ID NO: 16 - DNA, 5018 bp, artificial
  DoHu Dog
atggccctcggtgctctgcagagctgctccatccgccactcagagtcccagggaccccttccttcaaagtgtcggggcctgggtgatgggctgggcctctggagaggtgggcaggggccatctgaggtgaccagagtgggccatttgggcagcctgcaggctccagccgagcgattccagcacccgctctccttgggcttcgacgggaacccactctccaatatcttctcagcatccacgctgtacgagcattggcgggacaggagggtcttctggtgctgccgcctggggccgggtggccaggtgggccaggctgctggcgaggttgcgggaggggagcgggtgcgcatggagctctcagaggaagtgcacaggctgcttctgggaactgggcgtgctgcccaggaggggcaggcaggggagggggttggaagagcccgccgcacaccctcactggcgcacacagatgtgggtgtgcgcacaagtatgaacaaccgcgagcaggtgcccaaggggccctcgggcctgggcctgctcctgctcccccagctcctggctccacccagctcccctcttgcctccaacatgccccctgccccaaccctgggcattcggggcgagcccgtgtcccacgggcggccgaggagctcggccatcaggcctttctgccaaagccgtgacctccgtcagcgtgatgcccgggaggtacacgtacgcacatgcgtgcacacgcgcgtgcaagtgttgctcagcagcctggcccagagcctagcaaggagagcgcccagcccctcagcagccatcccgggagaaacccccgactcaggattcacggcccccagcaccacggccaggggccttgggggcattggcaagagggcccaggaccccggagagttggtgctggagacagagacgtgggggcaggtggttcaggggttagagccagccagcgccttcacttccggcctggtacgggccctgaggccctatgacgatgtccctgcatccagcttcaacagaggggagtctacagacccaggctgggaaaagccagctgtagtcggctatggctccccagccatcgtgggaacaacagggccggatctgactgccccccagggacaatcagcagccttgcggcaggaagcaatacggcgtgatgcaggaagctggggcccatttggggtccagtacgtggtctccatctggcctcagcgccttcgctctttggtggactcgggctggcgactgcacccttactccaaagacagctgggagagaagtgagggggcagtgccagccaggaccgtgaagctgcgccagcacaaaacccgcatcgtccgcagcacctctcctcctccagcctccttctttggggagaaccacctgcaggtgccggtgaccacagctctgagcaacatagacctccggctacaattctccacgtcccagcccgaagccctgctcctcctggcagcaggccaggctgaccacctcctcctgcagctccactccggatacctgcaggtcagactcaccctgggccaggaggagctgaggctgcagaccccagctgagactccgctgagcgactccgccgtccactccgtggagctgactgtgtcagacagcgaggcctcgttgtccgtcgatgggctgctgaacgcctcagcccccgtcctgggagctcccctggaggtcccctatgggatcttcctggggggcactgggagcctgagcctgtcctacctgatgggagccagccggcccctgaggggctgcctgcacgccgccaccgtcaacggccgcaacctcctccgaccactgacccctgacgtgcacgagggctgcgctgaagagttttctgctgatgacagcgtggctctgggcttctctgggccccactcgctggctgccttccctgcctggaacactcgggaggagggcaccctggcgttcatactcaccactcggagccgacaggcgcccctggctttccaggcgggcggccggcacggggatttcatctacgtggacatatttgagggccacctgcgggctgtggtggagaagggccagggcaccgtgttgctccacaacagcgtgcccgtggctgacgggctaccccatgaggtcagtgtccacgtggatgctcaccagctggaaatctccgtggaccagtaccccacacggacttccaaccgtgggatcctcagctacctggaaccccgcggcagtctcctcctgggggggctggacacagaggcctcccgccacctccaggaacaccgcctgggcctggcctcgggggccgtcaacgtctccctcctgggctgcatggaggatctcagcatcaacggccagaggcaggggctccgggaagcctcgctgactcgcagcatggtggccggctgcagcctggaggaagacgagtacgaggaggacacctacggcacctatgaagctctctccaccctggcaccggaggcctggtccgccgtggagctgcccgagccctgcgtgcccgaaccggggctgcctcccgtctttgccaacttcacccaactgctgactgtcagcccgctggtggtggccgaggggggcacagcctggcttgagtggcggcacctgcagcccacgctggacctgagcgaggccgagctgcgtaaatcccaggtgctgttcagcgtgagccgtggggcccgccacggggagctcgagctggacgtcccgggagcccaggcacggaaaatgttcaccctcctggacgtggtgaaccgcaaggcccgcttcgtccacgatggctcggaggagacctccgaccagctgatgctggaggtgtccgtgaccgccaggggccctgtgccctcctgcctccggaggggccagacttacatcctgcccatccagataaacccggtcaacgacccaccccaaatcatcttcccccacggcagcctcatggtgatcctggaacacacacagaagcccctggggcccgaggtcttccaggcctacgacccagactctgcctgcgagggcctcaccttccagctccttggcaccgccccgggcctgccggtggagcgccaggagcagcccggggagccagccaccgagttctcctgccgggagctggaggcgggcggcctggtctacgtgcaccggagcgggcccgcccaggacctgacgttccgcgtcagcgacgggctgcaggccagcgctccggccacgctgcaggtggtggcggtccggcccagcatccgggtccgccacaacacggggctgcgcctggcccagggctccgccgccccggtgctgcccgccaatctgtcggtggagaccaacgcggtggggcaggatgtgagcgtgctgttccgggtcgccgcggccctgcggttcggggagctgcagaagcagggcgcggggggcgccgagggcgcggagtggcgcccggtgcaggccttccagcagcgggacgtggagcagggccgcgtgaggtacctgagcaccgacccgcagcaccgcacggaggacgccgtggagcgcgtggccctggaggttcaggtgggccaggagaccctgagcaatctgtccttcctggtgacgatccagagagccaccgtgcggctgctgcggctcgagcccctgcgcacccacaccacgcggcaggaggcgctcaccggcgcgcacctggaggccgctctggaggagggggcgggccccagccccaccaccttccactacgagctggttcaggcccccaggaagggtaacctcaggctgcagggcgcccggctgtccgaggggcagggcttcacccaggatgacctgcaggccggccgggtgacctacggggccacggcgcgcacctcggagaccgtggaggacgccttccgtttccgcgtcacggctccgccacatttctccccgctctacaccttccccatccacatcgggggtgaccccgacgcccccgtcctcaccaacgtcctcctctccgtgcccgagggaggcgagggcgtcctctccgcggaacacctgttcgtcaagagcctcaacagcgccagctacctctatgaggtcatggagcggccccgccacgggcggctggtctggaggggggcgcaggacgaggccaccgcggtgacgtccttcaccaacgaggacctgctgcagggccggctggtctaccagcatgacaactccgagaccacggaagacgacatccccttcgtggcaacccgccagagtgagggcagcggcggcctggcctgggaggaggtccggggcgtcttccgcgtggccatccagcccgtgaacgaccacgctcccgtgcagaccgtcagccgcgtcttccacgtggcccggggcgggcggcggctgctgacgaccgacgacgtggccttcagtgacgccgactccggcttcgccgacgcgcagctggtgctgacccgcaaggaccttctcttcggcagcatcgtggccgcggacgagcccacgcggcccatctaccgcttctcccaggaggacctccggaagaggcgcgtcctgttcgtgcactccggggccgaccgcggctggatccagctgcaggtgtccgacgggcggcaccaggccaccgcgctgcttgaagtgcaggcatccgagccctatctccgcgtggccaatggctccagcctcgtggtccctcaggggggccagggcaccatcgacacagccgtgctccgcctggacaccaacctagacattcgcagcggggatgaggtccgctaccgtgtcacagccggcccgcactgggggcagctgctccgggccggccagccggccacagccttctcccaacaggacctgctggacggggccgtcctctacagccacaacggcagcctgagcccgcaggacaccctggccttctccgtggaggcagggcctgtgctcacggatgccaccctgcaggtgaccattgccttggaggggccattggccccactgcatctggtccagaacaagaa

SEQ ID NO: 17 - DNA, 3785 bp, artificial
  DoHux - Dog 3790
atgggctccccgcgctccggctccgcccggccccgccgacctgccgcgatgcggggtcagccgcccgcgcccccgggccccgcgctgcccctggccttggccttggctctgtgggcctgcgccgcctccgcggcctccttctttggggagaaccacctgcaggtgccggtgaccacagctctgagcaacatagacctccggctacaattctccacgtcccagcccgaagccctgctcctcctggcagcaggccaggctgaccacctcctcctgcagctccactccggatacctgcaggtcagactcaccctgggccaggaggagctgaggctgcagaccccagctgagactccgctgagcgactccgccgtccactccgtggagctgactgtgtcagacagcgaggcctcgttgtccgtcgatgggctgctgaacgcctcagcccccgtcctgggagctcccctggaggtcccctatgggatcttcctggggggcactgggagcctgagcctgtcctacctgatgggagccagccggcccctgaggggctgcctgcacgccgccaccgtcaacggccgcaacctcctccgaccactgacccctgacgtgcacgagggctgcgctgaagagttttctgctgatgacagcgtggctctgggcttctctgggccccactcgctggctgccttccctgcctggaacactcgggaggagggcaccctggcgttcatactcaccactcggagccgacaggcgcccctggctttccaggcgggcggccggcacggggatttcatctacgtggacatatttgagggccacctgcgggctgtggtggagaagggccagggcaccgtgttgctccacaacagcgtgcccgtggctgacgggctaccccatgaggtcagtgtccacgtggatgctcaccagctggaaatctccgtggaccagtaccccacacggacttccaaccgtgggatcctcagctacctggaaccccgcggcagtctcctcctgggggggctggacacagaggcctcccgccacctccaggaacaccgcctgggcctggcctcgggggccgtcaacgtctccctcctgggctgcatggaggatctcagcatcaacggccagaggcaggggctccgggaagcctcgctgactcgcagcatggtggccggctgcagcctggaggaagacgagtacgaggaggacacctacggcacctatgaagctctctccaccctggcaccggaggcctggtccgccgtggagctgcccgagccctgcgtgcccgaaccggggctgcctcccgtctttgccaacttcacccaactgctgactgtcagcccgctggtggtggccgaggggggcacagcctggcttgagtggcggcacctgcagcccacgctggacctgagcgaggccgagctgcgtaaatcccaggtgctgttcagcgtgagccgtggggcccgccacggggagctcgagctggacgtcccgggagcccaggcacggaaaatgttcaccctcctggacgtggtgaaccgcaaggcccgcttcgtccacgatggctcggaggagacctccgaccagctgatgctggaggtgtccgtgaccgccaggggccctgtgccctcctgcctccggaggggccagacttacatcctgcccatccagataaacccggtcaacgacccaccccaaatcatcttcccccacggcagcctcatggtgatcctggaacacacacagaagcccctggggcccgaggtcttccaggcctacgacccagactctgcctgcgagggcctcaccttccagctccttggcaccgccccgggcctgccggtggagcgccaggagcagcccggggagccagccaccgagttctcctgccgggagctggaggcgggcggcctggtctacgtgcaccggagcgggcccgcccaggacctgacgttccgcgtcagcgacgggctgcaggccagcgctccggccacgctgcaggtggtggcggtccggcccagcatccgggtccgccacaacacggggctgcgcctggcccagggctccgccgccccggtgctgcccgccaatctgtcggtggagaccaacgcggtggggcaggatgtgagcgtgctgttccgggtcgccgcggccctgcggttcggggagctgcagaagcagggcgcggggggcgccgagggcgcggagtggcgcccggtgcaggccttccagcagcgggacgtggagcagggccgcgtgaggtacctgagcaccgacccgcagcaccgcacggaggacgccgtggagcgcgtggccctggaggttcaggtgggccaggagaccctgagcaatctgtccttcctggtgacgatccagagagccaccgtgcggctgctgcggctcgagcccctgcgcacccacaccacgcggcaggaggcgctcaccggcgcgcacctggaggccgctctggaggagggggcgggccccagccccaccaccttccactacgagctggttcaggcccccaggaagggtaacctcaggctgcagggcgcccggctgtccgaggggcagggcttcacccaggatgacctgcaggccggccgggtgacctacggggccacggcgcgcacctcggagaccgtggaggacgccttccgtttccgcgtcacggctccgccacatttctccccgctctacaccttccccatccacatcgggggtgaccccgacgcccccgtcctcaccaacgtcctcctctccgtgcccgagggaggcgagggcgtcctctccgcggaacacctgttcgtcaagagcctcaacagcgccagctacctctatgaggtcatggagcggccccgccacgggcggctggtctggaggggggcgcaggacgaggccaccgcggtgacgtccttcaccaacgaggacctgctgcagggccggctggtctaccagcatgacaactccgagaccacggaagacgacatccccttcgtggcaacccgccagagtgagggcagcggcggcctggcctgggaggaggtccggggcgtcttccgcgtggccatccagcccgtgaacgaccacgctcccgtgcagaccgtcagccgcgtcttccacgtggcccggggcgggcggcggctgctgacgaccgacgacgtggccttcagtgacgccgactccggcttcgccgacgcgcagctggtgctgacccgcaaggaccttctcttcggcagcatcgtggccgcggacgagcccacgcggcccatctaccgcttctcccaggaggacctccggaagaggcgcgtcctgttcgtgcactccggggccgaccgcggctggatccagctgcaggtgtccgacgggcggcaccaggccaccgcgctgcttgaagtgcaggcatccgagccctatctccgcgtggccaatggctccagcctcgtggtccctcaggggggccagggcaccatcgacacagccgtgctccgcctggacaccaacctagacattcgcagcggggatgaggtccgctaccgtgtcacagccggcccgcactgggggcagctgctccgggccggccagccggccacagccttctcccaacaggacctgctggacggggccgtcctctacagccacaacggcagcctgagcccgcaggacaccctggccttctccgtggaggcagggcctgtgctcacggatgccaccctgcaggtgaccattgccttggaggggccattggccccactgcatctggtccagaacaagaa

SEQ ID NO: 18 - DNA, 5007 bp, artificial
  Dog D2+D3
cgcgtcagcgacgggctgcaggccagcgctccggccacgctgcaggtggtggcggtccggcccagcatccgggtccgccacaacacggggctgcgcctggcccagggctccgccgccccggtgctgcccgccaatctgtcggtggagaccaacgcggtggggcaggatgtgagcgtgctgttccgggtcgccgcggccctgcggttcggggagctgcagaagcagggcgcggggggcgccgagggcgcggagtggcgcccggtgcaggccttccagcagcgggacgtggagcagggccgcgtgaggtacctgagcaccgacccgcagcaccgcacggaggacgccgtggagcgcgtggccctggaggttcaggtgggccaggagaccctgagcaatctgtccttcctggtgacgatccagagagccaccgtgcggctgctgcggctcgagcccctgcgcacccacaccacgcggcaggaggcgctcaccggcgcgcacctggaggccgctctggaggagggggcgggccccagccccaccaccttccactacgagctggttcaggcccccaggaagggtaacctcaggctgcagggcgcccggctgtccgaggggcagggcttcacccaggatgacctgcaggccggccgggtgacctacggggccacggcgcgcacctcggagaccgtggaggacgccttccgtttccgcgtcacggctccgccacatttctccccgctctacaccttccccatccacatcgggggtgaccccgacgcccccgtcctcaccaacgtcctcctctccgtgcccgagggaggcgagggcgtcctctccgcggaacacctgttcgtcaagagcctcaacagcgccagctacctctatgaggtcatggagcggccccgccacgggcggctggtctggaggggggcgcaggacgaggccaccgcggtgacgtccttcaccaacgaggacctgctgcagggccggctggtctaccagcatgacaactccgagaccacggaagacgacatccccttcgtggcaacccgccagagtgagggcagcggcggcctggcctgggaggaggtccggggcgtcttccgcgtggccatccagcccgtgaacgaccacgctcccgtgcagaccgtcagccgcgtcttccacgtggcccggggcgggcggcggctgctgacgaccgacgacgtggccttcagtgacgccgactccggcttcgccgacgcgcagctggtgctgacccgcaaggaccttctcttcggcagcatcgtggccgcggacgagcccacgcggcccatctaccgcttctcccaggaggacctccggaagaggcgcgtcctgttcgtgcactccggggccgaccgcggctggatccagctgcaggtgtccgacgggcggcaccaggccaccgcgctgcttgaagtgcaggcatccgagccctatctccgcgtggccaatggctccagcctcgtggtccctcaggggggccagggcaccatcgacacagccgtgctccgcctggacaccaacctagacattcgcagcggggatgaggtccgctaccgtgtcacagccggcccgcactgggggcagctgctccgggccggccagccggccacagccttctcccaacaggacctgctggacggggccgtcctctacagccacaacggcagcctgagcccgcaggacaccctggccttctccgtggaggcagggcctgtgctcacggatgccaccctgcaggtgaccattgccttggaggggccattggccccactgcatctggtccagaacaagaagatctacgtcttccagggggaggcagctgagatcagaaaggatcagctggaggcagcgcaggaggcagtgccgcccgcccaaattgtgttctcggtgaagaccccgccgcgggccggctacctggtgatgctgtcccgcggcgcctccgtggccgggccgcccagctgggaccccgtgcagagcttctcccaggaggcggtggacgccggcagggtcctgtacctccactcccgccccgaggcctggagtgactccttctccctagacgtgggctcaggcctgggtgcgcccctcgagggcgtccgcgtggagctggaggtgctgcccgccaccatcccactggaggcacagaacttcagcgtccccgagggcggcagccgcgtgctggcccccccgctgctccaggtcgccgggccctacttccctgcactgcccggcctcgaactgcgggtcctcgagcagcccctgcacggggccctgcggagagaggaggcccctcaagcggggaccctcagcgctttctcctggaaagaggtagaacagcagcagatccgctatgtgcacgacgggagtgagacgctgacagacagcttcaccctagtggctaacgcctccgagctggaccgccagagccaccctgtggccttcaccatcaccgtcctgcccgtcaatgaccaaccgcccatcctcaccgcaaacacaggcctaacgatgtgggagggggccaccgtgcccttccctccggaggccctgaggggtgcggacagcgactcgggcccggaggacctggtctacaccatcgagcggcccagcaacgggcaggtggtgctgcgggcggcgccaggcaccgaggtgcacagcttcacgcaggcccagctggacgacgggctcgtgctgttctcacacagaggagccctggacggaggcttccgcttcagcctgtccgacggcgagcacgcttcccccggacacttcttccgcgtgacggcccagaagcagctgctcctctccctggagggcagccggacgctgaccgtgtgcccagggtcggtccagccgctcagcagccagagcctgagagccagctccagtgccggcaccgatccgcagcacctgctctaccgggtggtgcagggcccccggctgggccgcctgctccgcgcccagcagggcggcaccggggaggtcctggtgaacttcacgcaagccgaggtatacgcgggggatgttgtgtatgagcacaagatgcctgctgagcccttctgggaggtccacgacgccctggagctccggctgtcctcgccccccgcccccgacgtggccgccaccctggaggtggccgtgtccttcgaggccgcctgcccgcagcgccccagccgcctctggaggaacgagggtctctgggtggccgagggccagcaggcggacatcaccagcgccgccctggacgcctccaacctgctggcgcgcgtccccgccgcgctgcgcgcccggcacgacgtgctgttccaggtgacgcggttcccggcgcggggccggctgctgctggcggggcgggcgctgcacgcgggccgggcgcacttcctgcagtcggagctggcggcggggctcctggcctacgcgcacggcggcgggggcgcgcagcccgacggcttcggcttccgcgcgcagctgcagggccccgcgggcgccgggccgggcgcgctccccgcgctccccgcgctccccgacgaggccttcgccgtgcgcgtgggggccgcggcgtccgagccgctgcgcctgccccgcggctcccgcgcgcccgtgtcccgcgcgcagctccgcgtgcagctcccgggcgccgcgcccgccgacgtgcagtacgaggtgcggcgcgcggcccccggcggcttcctgagcctcgcgggcgcgggcgcgggcccggtgcgccgcttctcgcaggccgacgtggacgcgggccgcctggccttcgtggccaacggcagcagcgtggcgggcgtgctgcagctgagcgcgtgggccggcgccagcccgcgcgtgcccgtggcgctggccgtggacgtgctgcccgccgccatcgaggtgcagctgcgcgcgcccctggaggtgccccaggcgctggggcgctgcgcgctcgggccgcggcagctgcgcgtcgtgtcggaccgcgccgagcccgaggccgcctaccgcgtgacccgggcgccgcgcttcgggcagctcctggtggcgggcaggccggccggcgccttcagccagcggcaggtggaccgcggcgacgtggagttcgccttcaccgacctgtcctccccgcgcgaccgcttcgccgtcctggcccacgcgcggggcgccaacgccacggccacggtggacgtcacggtcgcggcgctgctgcgggtcgggccccgggggccgtggccgcagggcgccaccctgcgcctggacccggccgtcctggacgccgccgagctggccaaccgcacgggcggggagccgcgcttccgcctgctggccgggccccggctgggccgcctggtgcgcgtggcccgcgcggggccggagcccgtggagcagttcacgcagcgggacctggagggcgggaggctggggctgcagctgggccgcgcccccggccccacgggcgacagcctcacgctggagctgtgggcgcccggcgtccccccggccgtggcctccctggacttccacaccgagccctacgacgcggcgcgcccctacggcgtggccctgctcagcctccccgaggaagccggggcacccgacagcggcgccccggccacgggccagccgggcgcgccaggccccagccccgggcccaccgcggccagcggcggcttcctgggcctcctggaggccaacatgttcagcatcatcatccccgtgtgcctggtcctcctgctcctggccctgctcctgccgctgctcttctacctgcgcaagcggaacaagacgggcaagcacgacgtccaggtgctgaccgccaagccccgcaacggcctggccggcgacacggagaccttccgcaaggtggagccgggccacgccatcccgctcacggccgtgcccggccaggggcccccgcccggcggccagcccgacccagagctgctgcagtactgtcggacacccaaccccgccctcaaaaacggccagtactgggtgtga

SEQ ID NO: 19 - DNA, 2157 bp, artificial
  Dog D3
ctgaccgtgtgcccagggtcggtccagccgctcagcagccagagcctgagagccagctccagtgccggcaccgatccgcagcacctgctctaccgggtggtgcagggcccccggctgggccgcctgctccgcgcccagcagggcggcaccggggaggtcctggtgaacttcacgcaagccgaggtatacgcgggggatgttgtgtatgagcacaagatgcctgctgagcccttctgggaggtccacgacgccctggagctccggctgtcctcgccccccgcccccgacgtggccgccaccctggaggtggccgtgtccttcgaggccgcctgcccgcagcgccccagccgcctctggaggaacgagggtctctgggtggccgagggccagcaggcggacatcaccagcgccgccctggacgcctccaacctgctggcgcgcgtccccgccgcgctgcgcgcccggcacgacgtgctgttccaggtgacgcggttcccggcgcggggccggctgctgctggcggggcgggcgctgcacgcgggccgggcgcacttcctgcagtcggagctggcggcggggctcctggcctacgcgcacggcggcgggggcgcgcagcccgacggcttcggcttccgcgcgcagctgcagggccccgcgggcgccgggccgggcgcgctccccgcgctccccgcgctccccgacgaggccttcgccgtgcgcgtgggggccgcggcgtccgagccgctgcgcctgccccgcggctcccgcgcgcccgtgtcccgcgcgcagctccgcgtgcagctcccgggcgccgcgcccgccgacgtgcagtacgaggtgcggcgcgcggcccccggcggcttcctgagcctcgcgggcgcgggcgcgggcccggtgcgccgcttctcgcaggccgacgtggacgcgggccgcctggccttcgtggccaacggcagcagcgtggcgggcgtgctgcagctgagcgcgtgggccggcgccagcccgcgcgtgcccgtggcgctggccgtggacgtgctgcccgccgccatcgaggtgcagctgcgcgcgcccctggaggtgccccaggcgctggggcgctgcgcgctcgggccgcggcagctgcgcgtcgtgtcggaccgcgccgagcccgaggccgcctaccgcgtgacccgggcgccgcgcttcgggcagctcctggtggcgggcaggccggccggcgccttcagccagcggcaggtggaccgcggcgacgtggagttcgccttcaccgacctgtcctccccgcgcgaccgcttcgccgtcctggcccacgcgcggggcgccaacgccacggccacggtggacgtcacggtcgcggcgctgctgcgggtcgggccccgggggccgtggccgcagggcgccaccctgcgcctggacccggccgtcctggacgccgccgagctggccaaccgcacgggcggggagccgcgcttccgcctgctggccgggccccggctgggccgcctggtgcgcgtggcccgcgcggggccggagcccgtggagcagttcacgcagcgggacctggagggcgggaggctggggctgcagctgggccgcgcccccggccccacgggcgacagcctcacgctggagctgtgggcgcccggcgtccccccggccgtggcctccctggacttccacaccgagccctacgacgcggcgcgcccctacggcgtggccctgctcagcctccccgaggaagccggggcacccgacagcggcgccccggccacgggccagccgggcgcgccaggccccagccccgggcccaccgcggccagcggcggcttcctgggcctcctggaggccaacatgttcagcatcatcatccccgtgtgcctggtcctcctgctcctggccctgctcctgccgctgctcttctacctgcgcaagcggaacaagacgggcaagcacgacgtccaggtgctgaccgccaagccccgcaacggcctggccggcgacacggagaccttccgcaaggtggagccgggccacgccatcccgctcacggccgtgcccggccaggggcccccgcccggcggccagcccgacccagagctgctgcagtactgtcggacacccaaccccgccctcaaaaacggccagtactgggtgtga

SEQ ID NO: 20 - DNA, 5049 bp, artificial
  Human D2+D3
cgggtcagcgatggactgcaggccagccccccggccacgctgaaggtggtggccatccggccggccatacagatccaccgcagcacagggttgcgactggcccaaggctctgccatgcccatcttgcccgccaacctgtcggtggagaccaatgccgtggggcaggatgtgagcgtgctgttccgcgtcactggggccctgcagtttggggagctgcagaagcagggggcaggtggggtggagggtgctgagtggtgggccacacaggcgttccaccagcgggatgtggagcagggccgcgtgaggtacctgagcactgacccacagcaccacgcttacgacaccgtggagaacctggccctggaggtgcaggtgggccaggagatcctgagcaatctgtccttcccagtgaccatccagagagccactgtgtggatgctgcggctggagccactgcacactcagaacacccagcaggagaccctcaccacagcccacctggaggccaccctggaggaggcaggcccaagccccccaaccttccattatgaggtggttcaggctcccaggaaaggcaaccttcaactacagggcacaaggctgtcagatggccagggcttcacccaggatgacatacaggctggccgggtgacctatggggccacagcacgtgcctcagaggcagtcgaggacaccttccgtttccgtgtcacagctccaccatatttctccccactctataccttccccatccacattggtggtgacccagatgcgcctgtcctcaccaatgtcctcctcgtggtgcctgagggtggtgagggtgtcctctctgctgaccacctctttgtcaagagtctcaacagtgccagctacctctatgaggtcatggagcggccccgccatgggaggttggcttggcgtgggacacaggacaagaccactatggtgacatccttcaccaatgaagacctgttgcgtggccggctggtctaccagcatgatgactccgagaccacagaagatgatatcccatttgttgctacccgccagggcgagagcagtggtgacatggcctgggaggaggtacggggtgtcttccgagtggccatccagcccgtgaatgaccacgcccctgtgcagaccatcagccggatcttccatgtggcccggggtgggcggcggctgctgactacagacgacgtggccttcagcgatgctgactcgggctttgctgacgcccagctggtgcttacccgcaaggacctcctctttggcagtatcgtggccgtagatgagcccacgcggcccatctaccgcttcacccaggaggacctcaggaagaggcgagtactgttcgtgcactcaggggctgaccgtggctggatccagctgcaggtgtccgacgggcaacaccaggccactgcgctgctggaggtgcaggcctcggaaccctacctccgtgtggccaacggctccagccttgtggtccctcaaggaggccagggcaccatcgacacggccgtgctccacctggacaccaacctcgacatccgcagtggggatgaggtccactaccacgtcacagctggccctcgctggggacagctagtccgggctggtcagccagccacagccttctcccagcaggacctgctggatggggccgttctctatagccacaatggcagcctcagcccccgcgacaccatggccttctccgtggaagcagggccagtgcacacggatgccaccctacaagtgaccattgccctagagggcccactggccccactgaagctggtccggcacaagaagatctacgtcttccagggagaggcagctgagatcagaagggaccagctggaggcagcccaggaggcagtgccacctgcagacatcgtattctcagtgaagagcccaccgagtgccggctacctggtgatggtgtcgcgtggcgccttggcagatgagccacccagcctggaccctgtgcagagcttctcccaggaggcagtggacacaggcagggtcctgtacctgcactcccgccctgaggcctggagcgatgccttctcgctggatgtggcctcaggcctgggtgctcccctcgagggcgtccttgtggagctggaggtgctgcccgctgccatcccactagaggcgcaaaacttcagcgtccctgagggtggcagcctcaccctggcccctccactgctccgtgtctccgggccctacttccccactctcctgggcctcagcctgcaggtgctggagccaccccagcatggagccctgcagaaggaggacggacctcaagccaggaccctcagcgccttctcctggagaatggtggaagagcagctgatccgctacgtgcatgacgggagcgagacactgacagacagttttgtcctgatggctaatgcctccgagatggatcgccagagccatcctgtggccttcactgtcactgtcctgcctgtcaatgaccaaccccccatcctcactacaaacacaggcctgcagatgtgggagggggccactgcgcccatccctgcggaggctctgaggagcacggacggcgactctgggtctgaggatctggtctacaccatcgagcagcccagcaacgggcgggtagtgctgcggggggcgccgggcactgaggtgcgcagcttcacgcaggcccagctggacggcgggctcgtgctgttctcacacagaggaaccctggatggaggcttccgcttccgcctctctgacggcgagcacacttcccccggacacttcttccgagtgacggcccagaagcaagtgctcctctcgctgaagggcagccagacactgactgtctgcccagggtccgtccagccactcagcagtcagaccctcagggccagctccagcgcaggcactgacccccagctcctgctctaccgtgtggtgcggggcccccagctaggccggctgttccacgcccagcaggacagcacaggggaggccctggtgaacttcactcaggcagaggtctacgctgggaatattctgtatgagcatgagatgccccccgagcccttttgggaggcccatgataccctagagctccagctgtcctcgccgcctgcccgggacgtggccgccacccttgctgtggctgtgtcttttgaggctgcctgtccccagcgccccagccacctctggaagaacaaaggtctctgggtccccgagggccagcgggccaggatcaccgtggctgctctggatgcctccaatctcttggccagcgttccatcaccccagcgctcagagcatgatgtgctcttccaggtcacacagttccccagccggggccagctgttggtgtccgaggagcccctccatgctgggcagccccacttcctgcagtcccagctggctgcagggcagctagtgtatgcccacggcggtgggggcacccagcaggatggcttccactttcgtgcccacctccaggggccagcaggggcctccgtggctggaccccaaacctcagaggcctttgccatcacggtgagggatgtaaatgagcggccccctcagccacaggcctctgtcccactccggctcacccgaggctctcgtgcccccatctcccgggcccagctgagtgtggtggacccagactcagctcctggggagattgagtacgaggtccagcgggcaccccacaacggcttcctcagcctggtgggtggtggcctggggcccgtgacccgcttcacgcaagccgatgtggattcagggcggctggccttcgtggccaacgggagcagcgtggcaggcatcttccagctgagcatgtctgatggggccagcccacccctgcccatgtccctggctgtggacatcctaccatccgccatcgaggtgcagctgcgggcacccctggaggtgccccaagctttggggcgctcctcactgagccagcagcagctccgggtggtttcagatcgggaggagccagaggcagcataccgcctcatccagggaccccagtatgggcatctcctggtgggcgggcggcccacctcggccttcagccaattccagatagaccagggcgaggtggtctttgccttcaccaacttctcctcctctcatgaccacttcagagtcctggcactggctaggggtgtcaatgcatcagccgtagtgaacgtcactgtgagggctctgctgcatgtgtgggcaggtgggccatggccccagggtgccaccctgcgcctggaccccaccgtcctagatgctggcgagctggccaaccgcacaggcagtgtgccgcgcttccgcctcctggagggaccccggcatggccgcgtggtccgcgtgccccgagccaggacggagcccgggggcagccagctggtggagcagttcactcagcaggaccttgaggacgggaggctggggctggaggtgggcaggccagaggggagggcccccggccccgcaggtgacagtctcactctggagctgtgggcacagggcgtcccgcctgctgtggcctccctggactttgccactgagccttacaatgctgcccggccctacagcgtggccctgctcagtgtccccgaggccgcccggacggaagcagggaagccagagagcagcacccccacaggcgagccaggccccatggcatccagccctgagcccgctgtggccaagggaggcttcctgagcttccttgaggccaacatgttcagcgtcatcatccccatgtgcctggtacttctgctcctggcgctcatcctgcccctgctcttctacctccgaaaacgcaacaagacgggcaagcatgacgtccaggtcctgactgccaagccccgcaacggcctggctggtgacaccgagacctttcgcaaggtggagccaggccaggccatcccgctcacagctgtgcctggccaggggccccctccaggaggccagcctgacccagagctgctgcagttctgccggacacccaaccctgcccttaagaatggccagtactgggtgtga

SEQ ID NO: 21 - DNA, 2202 bp, artificial
  Human D3
ctgactgtctgcccagggtccgtccagccactcagcagtcagaccctcagggccagctccagcgcaggcactgacccccagctcctgctctaccgtgtggtgcggggcccccagctaggccggctgttccacgcccagcaggacagcacaggggaggccctggtgaacttcactcaggcagaggtctacgctgggaatattctgtatgagcatgagatgccccccgagcccttttgggaggcccatgataccctagagctccagctgtcctcgccgcctgcccgggacgtggccgccacccttgctgtggctgtgtcttttgaggctgcctgtccccagcgccccagccacctctggaagaacaaaggtctctgggtccccgagggccagcgggccaggatcaccgtggctgctctggatgcctccaatctcttggccagcgttccatcaccccagcgctcagagcatgatgtgctcttccaggtcacacagttccccagccggggccagctgttggtgtccgaggagcccctccatgctgggcagccccacttcctgcagtcccagctggctgcagggcagctagtgtatgcccacggcggtgggggcacccagcaggatggcttccactttcgtgcccacctccaggggccagcaggggcctccgtggctggaccccaaacctcagaggcctttgccatcacggtgagggatgtaaatgagcggccccctcagccacaggcctctgtcccactccggctcacccgaggctctcgtgcccccatctcccgggcccagctgagtgtggtggacccagactcagctcctggggagattgagtacgaggtccagcgggcaccccacaacggcttcctcagcctggtgggtggtggcctggggcccgtgacccgcttcacgcaagccgatgtggattcagggcggctggccttcgtggccaacgggagcagcgtggcaggcatcttccagctgagcatgtctgatggggccagcccacccctgcccatgtccctggctgtggacatcctaccatccgccatcgaggtgcagctgcgggcacccctggaggtgccccaagctttggggcgctcctcactgagccagcagcagctccgggtggtttcagatcgggaggagccagaggcagcataccgcctcatccagggaccccagtatgggcatctcctggtgggcgggcggcccacctcggccttcagccaattccagatagaccagggcgaggtggtctttgccttcaccaacttctcctcctctcatgaccacttcagagtcctggcactggctaggggtgtcaatgcatcagccgtagtgaacgtcactgtgagggctctgctgcatgtgtgggcaggtgggccatggccccagggtgccaccctgcgcctggaccccaccgtcctagatgctggcgagctggccaaccgcacaggcagtgtgccgcgcttccgcctcctggagggaccccggcatggccgcgtggtccgcgtgccccgagccaggacggagcccgggggcagccagctggtggagcagttcactcagcaggaccttgaggacgggaggctggggctggaggtgggcaggccagaggggagggcccccggccccgcaggtgacagtctcactctggagctgtgggcacagggcgtcccgcctgctgtggcctccctggactttgccactgagccttacaatgctgcccggccctacagcgtggccctgctcagtgtccccgaggccgcccggacggaagcagggaagccagagagcagcacccccacaggcgagccaggccccatggcatccagccctgagcccgctgtggccaagggaggcttcctgagcttccttgaggccaacatgttcagcgtcatcatccccatgtgcctggtacttctgctcctggcgctcatcctgcccctgctcttctacctccgaaaacgcaacaagacgggcaagcatgacgtccaggtcctgactgccaagccccgcaacggcctggctggtgacaccgagacctttcgcaaggtggagccaggccaggccatcccgctcacagctgtgcctggccaggggccccctccaggaggccagcctgacccagagctgctgcagttctgccggacacccaaccctgcccttaagaatggccagtactgggtgtga

SEQ ID NO: 22 - DNA, 3187 bp, artificial
  HuDo Dog
gatctacgtcttccagggggaggcagctgagatcagaaaggatcagctggaggcagcgcaggaggcagtgccgcccgcccaaattgtgttctcggtgaagaccccgccgcgggccggctacctggtgatgctgtcccgcggcgcctccgtggccgggccgcccagctgggaccccgtgcagagcttctcccaggaggcggtggacgccggcagggtcctgtacctccactcccgccccgaggcctggagtgactccttctccctagacgtgggctcaggcctgggtgcgcccctcgagggcgtccgcgtggagctggaggtgctgcccgccaccatcccactggaggcacagaacttcagcgtccccgagggcggcagccgcgtgctggcccccccgctgctccaggtcgccgggccctacttccctgcactgcccggcctcgaactgcgggtcctcgagcagcccctgcacggggccctgcggagagaggaggcccctcaagcggggaccctcagcgctttctcctggaaagaggtagaacagcagcagatccgctatgtgcacgacgggagtgagacgctgacagacagcttcaccctagtggctaacgcctccgagctggaccgccagagccaccctgtggccttcaccatcaccgtcctgcccgtcaatgaccaaccgcccatcctcaccgcaaacacaggcctaacgatgtgggagggggccaccgtgcccttccctccggaggccctgaggggtgcggacagcgactcgggcccggaggacctggtctacaccatcgagcggcccagcaacgggcaggtggtgctgcgggcggcgccaggcaccgaggtgcacagcttcacgcaggcccagctggacgacgggctcgtgctgttctcacacagaggagccctggacggaggcttccgcttcagcctgtccgacggcgagcacgcttcccccggacacttcttccgcgtgacggcccagaagcagctgctcctctccctggagggcagccggacgctgaccgtgtgcccagggtcggtccagccgctcagcagccagagcctgagagccagctccagtgccggcaccgatccgcagcacctgctctaccgggtggtgcagggcccccggctgggccgcctgctccgcgcccagcagggcggcaccggggaggtcctggtgaacttcacgcaagccgaggtatacgcgggggatgttgtgtatgagcacaagatgcctgctgagcccttctgggaggtccacgacgccctggagctccggctgtcctcgccccccgcccccgacgtggccgccaccctggaggtggccgtgtccttcgaggccgcctgcccgcagcgccccagccgcctctggaggaacgagggtctctgggtggccgagggccagcaggcggacatcaccagcgccgccctggacgcctccaacctgctggcgcgcgtccccgccgcgctgcgcgcccggcacgacgtgctgttccaggtgacgcggttcccggcgcggggccggctgctgctggcggggcgggcgctgcacgcgggccgggcgcacttcctgcagtcggagctggcggcggggctcctggcctacgcgcacggcggcgggggcgcgcagcccgacggcttcggcttccgcgcgcagctgcagggccccgcgggcgccgggccgggcgcgctccccgcgctccccgcgctccccgacgaggccttcgccgtgcgcgtgggggccgcggcgtccgagccgctgcgcctgccccgcggctcccgcgcgcccgtgtcccgcgcgcagctccgcgtgcagctcccgggcgccgcgcccgccgacgtgcagtacgaggtgcggcgcgcggcccccggcggcttcctgagcctcgcgggcgcgggcgcgggcccggtgcgccgcttctcgcaggccgacgtggacgcgggccgcctggccttcgtggccaacggcagcagcgtggcgggcgtgctgcagctgagcgcgtgggccggcgccagcccgcgcgtgcccgtggcgctggccgtggacgtgctgcccgccgccatcgaggtgcagctgcgcgcgcccctggaggtgccccaggcgctggggcgctgcgcgctcgggccgcggcagctgcgcgtcgtgtcggaccgcgccgagcccgaggccgcctaccgcgtgacccgggcgccgcgcttcgggcagctcctggtggcgggcaggccggccggcgccttcagccagcggcaggtggaccgcggcgacgtggagttcgccttcaccgacctgtcctccccgcgcgaccgcttcgccgtcctggcccacgcgcggggcgccaacgccacggccacggtggacgtcacggtcgcggcgctgctgcgggtcgggccccgggggccgtggccgcagggcgccaccctgcgcctggacccggccgtcctggacgccgccgagctggccaaccgcacgggcggggagccgcgcttccgcctgctggccgggccccggctgggccgcctggtgcgcgtggcccgcgcggggccggagcccgtggagcagttcacgcagcgggacctggagggcgggaggctggggctgcagctgggccgcgcccccggccccacgggcgacagcctcacgctggagctgtgggcgcccggcgtccccccggccgtggcctccctggacttccacaccgagccctacgacgcggcgcgcccctacggcgtggccctgctcagcctccccgaggaagccggggcacccgacagcggcgccccggccacgggccagccgggcgcgccaggccccagccccgggcccaccgcggccagcggcggcttcctgggcctcctggaggccaacatgttcagcatcatcatccccgtgtgcctggtcctcctgctcctggccctgctcctgccgctgctcttctacctgcgcaagcggaacaagacgggcaagcacgacgtccaggtgctgaccgccaagccccgcaacggcctggccggcgacacggagaccttccgcaaggtggagccgggccacgccatcccgctcacggccgtgcccggccaggggcccccgcccggcggccagcccgacccagagctgctgcagtactgtcggacacccaaccccgccctcaaaaacggccagtactgggtgtag

SEQ ID NO: 23 - DNA, 3232 bp, artificial
  DoHu Hu
gatctacgtcttccagggagaggcagctgagatcagaagggaccagctggaggcagcccaggaggcagtgccacctgcagacatcgtattctcagtgaagagcccaccgagtgccggctacctggtgatggtgtcgcgtggcgccttggcagatgagccacccagcctggaccctgtgcagagcttctcccaggaggcagtggacacaggcagggtcctgtacctgcactcccgccctgaggcctggagcgatgccttctcgctggatgtggcctcaggcctgggtgctcccctcgagggcgtccttgtggagctggaggtgctgcccgctgccatcccactagaggcgcaaaacttcagcgtccctgagggtggcagcctcaccctggcccctccactgctccgtgtctccgggccctacttccccactctcctgggcctcagcctgcaggtgctggagccaccccagcatggagccctgcagaaggaggacggacctcaagccaggaccctcagcgccttctcctggagaatggtggaagagcagctgatccgctacgtgcatgacgggagcgagacactgacagacagttttgtcctgatggctaatgcctccgagatggatcgccagagccatcctgtggccttcactgtcactgtcctgcctgtcaatgaccaaccccccatcctcactacaaacacaggcctgcagatgtgggagggggccactgcgcccatccctgcggaggctctgaggagcacggacggcgactctgggtctgaggatctggtctacaccatcgagcagcccagcaacgggcgggtagtgctgcggggggcgccgggcactgaggtgcgcagcttcacgcaggcccagctggacggcgggctcgtgctgttctcacacagaggaaccctggatggaggcttccgcttccgcctctctgacggcgagcacacttcccccggacacttcttccgagtgacggcccagaagcaagtgctcctctcgctgaagggcagccagacactgactgtctgcccagggtccgtccagccactcagcagtcagaccctcagggccagctccagcgcaggcactgacccccagctcctgctctaccgtgtggtgcggggcccccagctaggccggctgttccacgcccagcaggacagcacaggggaggccctggtgaacttcactcaggcagaggtctacgctgggaatattctgtatgagcatgagatgccccccgagcccttttgggaggcccatgataccctagagctccagctgtcctcgccgcctgcccgggacgtggccgccacccttgctgtggctgtgtcttttgaggctgcctgtccccagcgccccagccacctctggaagaacaaaggtctctgggtccccgagggccagcgggccaggatcaccgtggctgctctggatgcctccaatctcttggccagcgttccatcaccccagcgctcagagcatgatgtgctcttccaggtcacacagttccccagccggggccagctgttggtgtccgaggagcccctccatgctgggcagccccacttcctgcagtcccagctggctgcagggcagctagtgtatgcccacggcggtgggggcacccagcaggatggcttccactttcgtgcccacctccaggggccagcaggggcctccgtggctggaccccaaacctcagaggcctttgccatcacggtgagggatgtaaatgagcggccccctcagccacaggcctctgtcccactccggctcacccgaggctctcgtgcccccatctcccgggcccagctgagtgtggtggacccagactcagctcctggggagattgagtacgaggtccagcgggcaccccacaacggcttcctcagcctggtgggtggtggcctggggcccgtgacccgcttcacgcaagccgatgtggattcagggcggctggccttcgtggccaacgggagcagcgtggcaggcatcttccagctgagcatgtctgatggggccagcccacccctgcccatgtccctggctgtggacatcctaccatccgccatcgaggtgcagctgcgggcacccctggaggtgccccaagctttggggcgctcctcactgagccagcagcagctccgggtggtttcagatcgggaggagccagaggcagcataccgcctcatccagggaccccagtatgggcatctcctggtgggcgggcggcccacctcggccttcagccaattccagatagaccagggcgaggtggtctttgccttcaccaacttctcctcctctcatgaccacttcagagtcctggcactggctaggggtgtcaatgcatcagccgtagtgaacgtcactgtgagggctctgctgcatgtgtgggcaggtgggccatggccccagggtgccaccctgcgcctggaccccaccgtcctagatgctggcgagctggccaaccgcacaggcagtgtgccgcgcttccgcctcctggagggaccccggcatggccgcgtggtccgcgtgccccgagccaggacggagcccgggggcagccagctggtggagcagttcactcagcaggaccttgaggacgggaggctggggctggaggtgggcaggccagaggggagggcccccggccccgcaggtgacagtctcactctggagctgtgggcacagggcgtcccgcctgctgtggcctccctggactttgccactgagccttacaatgctgcccggccctacagcgtggccctgctcagtgtccccgaggccgcccggacggaagcagggaagccagagagcagcacccccacaggcgagccaggccccatggcatccagccctgagcccgctgtggccaagggaggcttcctgagcttccttgaggccaacatgttcagcgtcatcatccccatgtgcctggtacttctgctcctggcgctcatcctgcccctgctcttctacctccgaaaacgcaacaagacgggcaagcatgacgtccaggtcctgactgccaagccccgcaacggcctggctggtgacaccgagacctttcgcaaggtggagccaggccaggccatcccgctcacagctgtgcctggccaggggccccctccaggaggccagcctgacccagagctgctgcagttctgccggacacccaaccctgcccttaagaatggccagtactgggtgtga